European Patent Application EP 4 682 172 A1, published January 21, 2026. Title: ANTI-MUC17, ANTI-CD3 AND ANTI-CD28 TRISPECIFIC ANTIBODY. Applicant: ANTI-MUC17, ANTI-CD3 AND ANTI-CD28 TRISPECIFIC ANTIBODY. The sequence listing filed with the application follows.

SEQUENCE LISTING (53 sequences)

SEQ ID NO: 1 - protein, 121 aa, synthetic construct
  source 1..121: note = Amino acid sequence of VH of murine monoclonal antibody 44H4 against MUC17
EVQLQQSGAELVKPGASVKLSFTASGFNIKDTYIHWVKQRPEQGLEWIGRIDPANGYTKYGPRFQGKATITADTASNAAYLQLSSLTSEDTAVYYCARNYGTSYPNAMDYWGQGTSVTVSS

SEQ ID NO: 2 - protein, 111 aa, synthetic construct
  source 1..111: note = Amino acid sequence of VL of murine monoclonal antibody 44H4 against MUC17
DIVLTQSPASLAVSLGQRATISCRASESVETYGNSFMHWYQQKPGQPPKLLIYRASSLESGIPARFSGSGSRTDFTLTITPVEADDVATYFCQQSNEDPYTFGGGTKLEIK

SEQ ID NO: 3 - protein, 5 aa, synthetic construct
  source 1..5: note = H-CDR1 of murine monoclonal antibody 44H4
DTYIH

SEQ ID NO: 4 - protein, 17 aa, synthetic construct
  source 1..17: note = H-CDR2 of murine monoclonal antibody 44H4
RIDPANGYTKYGPRFQG

SEQ ID NO: 5 - protein, 12 aa, synthetic construct
  source 1..12: note = H-CDR3 of murine monoclonal antibody 44H4
NYGTSYPNAMDY

SEQ ID NO: 6 - protein, 15 aa, synthetic construct
  source 1..15: note = L-CDR1 of murine monoclonal antibody 44H4
RASESVETYGNSFMH

SEQ ID NO: 7 - protein, 7 aa, synthetic construct
  source 1..7: note = L-CDR2 of murine monoclonal antibody 44H4
RASSLES

SEQ ID NO: 8 - protein, 9 aa, synthetic construct
  source 1..9: note = L-CDR3 of murine monoclonal antibody 44H4
QQSNEDPYT

SEQ ID NO: 9 - protein, 121 aa, synthetic construct
  source 1..121: note = Amino acid sequence of VH of 44H4 humanized antibody
QVQLVQSGAEVKKPGASVKVSCKASGFNIKDTYIHWVRQAPGQGLEWMGRIDPANGYTKYGPRFQGRVTITADTSTSTVYMELSSLRSEDTAVYYCARNYGTSYPNAMDYWGQGTLVTVSS

SEQ ID NO: 10 - protein, 111 aa, synthetic construct
  source 1..111: note = Amino acid sequence of VL of 44H4 humanized antibody
DIVLTQSPASLAVSPGQRATITCRASESVETYGNSFMHWYQQKPGQPPKLLIYRASSLESGVPARFSGSGSGTDFTLTINPVEADDTANYYCQQSNEDPYTFGQGTKVEIK

SEQ ID NO: 11 - protein, 330 aa, synthetic construct
  source 1..330: note = Amino acid sequence of human IgG1 heavy chain constant region
ASTKGPSVFPLAPSSKSTSGGTAALGCLVKDYFPEPVTVSWNSGALTSGVHTFPAVLQSSGLYSLSSVVTVPSSSLGTQTYICNVNHKPSNTKVDKKVEPKSCDKTHTCPPCPAPELLGGPSVFLFPPKPKDTLMISRTPEVTCVVVDVSHEDPEVKFNWYVDGVEVHNAKTKPREEQYNSTYRVVSVLTVLHQDWLNGKEYKCKVSNKALPAPIEKTISKAKGQPREPQVYTLPPSREEMTKNQVSLTCLVKGFYPSDIAVEWESNGQPENNYKTTPPVLDSDGSFFLYSKLTVDKSRWQQGNVFSCSVMHEALHNHYTQKSLSLSPGK

SEQ ID NO: 12 - protein, 451 aa, synthetic construct
  source 1..451: note = Amino acid sequence of 44H4-Hu-HC
QVQLVQSGAEVKKPGASVKVSCKASGFNIKDTYIHWVRQAPGQGLEWMGRIDPANGYTKYGPRFQGRVTITADTSTSTVYMELSSLRSEDTAVYYCARNYGTSYPNAMDYWGQGTLVTVSSASTKGPSVFPLAPSSKSTSGGTAALGCLVKDYFPEPVTVSWNSGALTSGVHTFPAVLQSSGLYSLSSVVTVPSSSLGTQTYICNVNHKPSNTKVDKKVEPKSCDKTHTCPPCPAPELLGGPSVFLFPPKPKDTLMISRTPEVTCVVVDVSHEDPEVKFNWYVDGVEVHNAKTKPREEQYNSTYRVVSVLTVLHQDWLNGKEYKCKVSNKALPAPIEKTISKAKGQPREPQVYTLPPSREEMTKNQVSLTCLVKGFYPSDIAVEWESNGQPENNYKTTPPVLDSDGSFFLYSKLTVDKSRWQQGNVFSCSVMHEALHNHYTQKSLSLSPGK

SEQ ID NO: 13 - protein, 107 aa, synthetic construct [sequence omitted]

SEQ ID NO: 14 - protein, 218 aa, synthetic construct
  source 1..218: note = Amino acid sequence of 44H4-Hu-LC
DIVLTQSPASLAVSPGQRATITCRASESVETYGNSFMHWYQQKPGQPPKLLIYRASSLESGVPARFSGSGSGTDFTLTINPVEADDTANYYCQQSNEDPYTFGQGTKVEIKRTVAAPSVFIFPPSDEQLKSGTASVVCLLNNFYPREAKVQWKVDNALQSGNSQESVTEQDSKDSTYSLSSTLTLSKADYEKHKVYACEVTHQGLSSPVTKSFNRGEC

SEQ ID NO: 15 - protein, 125 aa, synthetic construct
  source 1..125: note = Amino acid sequence of VH of SP34 antibody
EVKLLESGGGLVQPKGSLKLSCAASGFTFNTYAMNWVRQAPGKGLEWVARIRSKYNNYATYYADSVKDRFTISRDDSQSILYLQMNNLKTEDTAMYYCVRHGNFGNSYVSWFAYWGQGTLVTVSA

SEQ ID NO: 16 - protein, 109 aa, synthetic construct
  source 1..109: note = Amino acid sequence of VL of SP34 antibody
QAVVTQESALTTSPGETVTLTCRSSTGAVTTSNYANWVQEKPDHLFTGLIGGTNKRAPGVPARFSGSLIGDKAALTITGAQTEDEAIYFCALWYSNLWVFGGGTKLTVL

SEQ ID NO: 17 - protein, 5 aa, synthetic construct
  source 1..5: note = H-CDR1 of SP34 antibody
TYAMN

SEQ ID NO: 18 - protein, 19 aa, synthetic construct
  source 1..19: note = H-CDR2 of SP34 antibody
RIRSKYNNYATYYADSVKD

SEQ ID NO: 19 - protein, 14 aa, synthetic construct
  source 1..14: note = H-CDR3 of SP34 antibody
HGNFGNSYVSWFAY

SEQ ID NO: 20 - protein, 14 aa, synthetic construct
  source 1..14: note = L-CDR1 of SP34 antibody
RSSTGAVTTSNYAN

SEQ ID NO: 21 - protein, 7 aa, synthetic construct
  source 1..7: note = L-CDR2 of SP34 antibody
GTNKRAP

SEQ ID NO: 22 - protein, 9 aa, synthetic construct
  source 1..9: note = L-CDR3 of SP34 antibody
ALWYSNLWV

SEQ ID NO: 23 - protein, 125 aa, synthetic construct
  source 1..125: note = Amino acid sequence of VH of SP34 humanized antibody
EVQLVESGGGLVQPGGSLRLSCAASGFTFSTYAMNWVRQAPGKGLEWVSRIRSKYNNYATYYADSVKDRFTISRDDSKNTLYLQMNSLRAEDTAVYYCARHDNFGNSYVSWFAYWGQGTLVTVSS

SEQ ID NO: 24 - protein, 109 aa, synthetic construct
  source 1..109: note = Amino acid sequence of VL of SP34 humanized antibody
QTVVTQEPSLTVSPGGTVTLTCGSSTGAVTTSNYPNWVQQKPGQAPRGLIGGTNKRAPGVPARFSGSLLGGKAALTLSGAQPEDEAEYYCALWYSDLWVFGGGTKLTVL

SEQ ID NO: 25 - protein, 455 aa, synthetic construct
  source 1..455: note = Amino acid sequence of SP34-Hu-HC
EVQLVESGGGLVQPGGSLRLSCAASGFTFSTYAMNWVRQAPGKGLEWVSRIRSKYNNYATYYADSVKDRFTISRDDSKNTLYLQMNSLRAEDTAVYYCARHDNFGNSYVSWFAYWGQGTLVTVSSASTKGPSVFPLAPSSKSTSGGTAALGCLVKDYFPEPVTVSWNSGALTSGVHTFPAVLQSSGLYSLSSVVTVPSSSLGTQTYICNVNHKPSNTKVDKKVEPKSCDKTHTCPPCPAPELLGGPSVFLFPPKPKDTLMISRTPEVTCVVVDVSHEDPEVKFNWYVDGVEVHNAKTKPREEQYNSTYRVVSVLTVLHQDWLNGKEYKCKVSNKALPAPIEKTISKAKGQPREPQVYTLPPSREEMTKNQVSLTCLVKGFYPSDIAVEWESNGQPENNYKTTPPVLDSDGSFFLYSKLTVDKSRWQQGNVFSCSVMHEALHNHYTQKSLSLSPGK

SEQ ID NO: 26 - protein, 106 aa, synthetic construct
  source 1..106: note = Amino acid sequence of lambda light chain constant region
GQPKAAPSVTLFPPSSEELQANKATLVCLISDFYPGAVTVAWKADSSPVKAGVETTTPSKQSNNKYAASSYLSLTPEQWKSHRSYSCQVTHEGSTVEKTVAPTECS

SEQ ID NO: 27 - protein, 215 aa, synthetic construct
  source 1..215: note = Amino acid sequence of SP34-Hu-LC
QTVVTQEPSLTVSPGGTVTLTCGSSTGAVTTSNYPNWVQQKPGQAPRGLIGGTNKRAPGVPARFSGSLLGGKAALTLSGAQPEDEAEYYCALWYSDLWVFGGGTKLTVLGQPKAAPSVTLFPPSSEELQANKATLVCLISDFYPGAVTVAWKADSSPVKAGVETTTPSKQSNNKYAASSYLSLTPEQWKSHRSYSCQVTHEGSTVEKTVAPTECS

SEQ ID NO: 28 - protein, 120 aa, synthetic construct
  source 1..120: note = Amino acid sequence of VH of anti-CD28
QVQLVQSGAEVKKPGASVKVSCKASGYTFTSYYIHWVRQAPGQGLEWIGCIYPGNVNTNYNEKFKDRATLTVDTSISTAYMELSRLRSDDTAVYFCTRSHYGLDWNFDVWGQGTTVTVSS

SEQ ID NO: 29 - protein, 107 aa, synthetic construct
  source 1..107: note = Amino acid sequence of VL of anti-CD28
DIQMTQSPSSLSASVGDRVTITCHASQNIYVWLNWYQQKPGKAPKLLIYKASNLHTGVPSRFSGSGSGTDFTLTISSLQPEDFATYYCQQGQTYPYTFGGGTKVEIK

SEQ ID NO: 30 - protein, 5 aa, synthetic construct
  source 1..5: note = H-CDR1 of Anti-CD28 antibody
SYYIH

SEQ ID NO: 31 - protein, 17 aa, synthetic construct
  source 1..17: note = H-CDR2 of Anti-CD28 antibody
CIYPGNVNTNYNEKFKD

SEQ ID NO: 32 - protein, 11 aa, synthetic construct
  source 1..11: note = H-CDR3 of Anti-CD28 antibody
SHYGLDWNFDV

SEQ ID NO: 33 - protein, 11 aa, synthetic construct
  source 1..11: note = L-CDR1 of Anti-CD28 antibody
HASQNIYVWLN

SEQ ID NO: 34 - protein, 7 aa, synthetic construct
  source 1..7: note = L-CDR2 of Anti-CD28 antibody
KASNLHT

SEQ ID NO: 35 - protein, 9 aa, synthetic construct
  source 1..9: note = L-CDR3 of Anti-CD28 antibody
QQGQTYPYT

SEQ ID NO: 36 - protein, 450 aa, synthetic construct
  source 1..450: note = Amino acid sequence of anti-CD28-Hu-HC
QVQLVQSGAEVKKPGASVKVSCKASGYTFTSYYIHWVRQAPGQGLEWMGSIYPGNVNTNYNEKFKDRVTLTVDTSISTAYMELSRLRSDDTAVYYCTRSHYGLDWNFDVWGQGTTVTVSSASTKGPSVFPLAPSSKSTSGGTAALGCLVKDYFPEPVTVSWNSGALTSGVHTFPAVLQSSGLYSLSSVVTVPSSSLGTQTYICNVNHKPSNTKVDKKVEPKSCDKTHTCPPCPAPELLGGPSVFLFPPKPKDTLMISRTPEVTCVVVDVSHEDPEVKFNWYVDGVEVHNAKTKPREEQYNSTYRVVSVLTVLHQDWLNGKEYKCKVSNKALPAPIEKTISKAKGQPREPQVYTLPPSREEMTKNQVSLTCLVKGFYPSDIAVEWESNGQPENNYKTTPPVLDSDGSFFLYSKLTVDKSRWQQGNVFSCSVMHEALHNHYTQKSLSLSPGK

SEQ ID NO: 37 - protein, 214 aa, synthetic construct
  source 1..214: note = Amino acid sequence of anti-CD28-Hu-LC
DIQMTQSPSSLSASVGDRVTITCHASQNIYVWLNWYQQKPGKAPKLLIYKASNLHTGVPSRFSGSGSGTDFTLTISSLQPEDFATYYCQQGQTYPYTFGGGTKVEIKRTVAAPSVFIFPPSDEQLKSGTASVVCLLNNFYPREAKVQWKVDNALQSGNSQESVTEQDSKDSTYSLSSTLTLSKADYEKHKVYACEVTHQGLSSPVTKSFNRGEC

SEQ ID NO: 38 - protein, 733 aa, synthetic construct
  source 1..733: note = Amino acid sequence of CD28-44-SP34-Dia-IgG1-Knob-HC
DIQMTQSPSSLSASVGDRVTITCHASQNIYVWLNWYQQKPGKAPKLLIYKASNLHTGVPSRFSGSGSGTDFTLTISSLQPEDFATYYCQQGQTYPYTFGCGTKVEIKGGGGSEVQLVESGGGLVQPGGSLRLSCAASGFTFSTYAMNWVRQAPGKGLEWVSRIRSKYNNYATYYADSVKDRFTISRDDSKNTLYLQMNSLRAEDTAVYYCARHDNFGNSYVSWFAYWGQGTLVTVSSGGGGSGGGGSGGGGSGGGGSQTVVTQEPSLTVSPGGTVTLTCGSSTGAVTTSNYPNWVQQKPGQAPRGLIGGTNKRAPGVPARFSGSLLGGKAALTLSGAQPEDEAEYYCALWYSDLWVFGGGTKLTVLGGGGSQVQLVQSGAEVKKPGASVKVSCKASGYTFTSYYIHWVRQAPGQCLEWMGSIYPGNVNTNYNEKFKDRVTLTVDTSISTAYMELSRLRSDDTAVYYCTRSHYGLDWNFDVWGQGTTVTVSSGGGGSGGGGSGGGGSDKTHTCPPCPAPEAAGAPSVFLFPPKPKDTLMISRTPEVTCVVVDVSHEDPEVKFNWYVDGVEVHNAKTKPREEQYNSTYRVVSVLTVLHQDWLNGKEYKCKVSNKALPAPIEKTISKAKGQPREPQVYTLPPCRDELTKNQVSLWCLVKGFYPSDIAVEWESNGQPENNYKTTPPVLDSDGSFFLYSKLTVDKSRWQQGNVFSCSVMHEALHNHYTQKSLSLSPGK

SEQ ID NO: 39 - protein, 2199 aa, synthetic construct
  source 1..2199: note = Nucleotide sequence of CD28-44-SP34-Dia-IgG1-Knob-HC
GACATCCAGATGACCCAGAGTCCCAGCAGCCTGTCTGCTTCTGTGGGAGATAGAGTGACAATTACATGTCATGCTTCTCAGAATATCTACGTGTGGCTGAACTGGTACCAGCAGAAACCTGGAAAGGCTCCTAAGCTGCTGATCTACAAGGCTTCTAACCTGCACACAGGCGTGCCTTCTAGATTTTCTGGATCTGGCTCCGGAACAGATTTTACTCTGACCATCTCTAGCCTGCAGCCAGAAGATTTTGCCACCTATTATTGTCAGCAGGGACAGACCTACCCTTACACATTTGGCTGCGGCACAAAGGTGGAGATCAAGGGTGGAGGCGGTAGCGAGGTGCAGCTGGTGGAGTCTGGCGGCGGCCTGGTGCAGCCTGGCGGCTCTCTGAGACTGTCTTGTGCTGCTTCTGGCTTTACCTTTTCTACCTATGCTATGAATTGGGTGAGACAGGCTCCTGGCAAGGGCCTGGAGTGGGTGTCTAGAATCAGATCTAAGTATAATAATTACGCTACCTATTATGCTGATTCTGTGAAGGACAGATTCACAATCTCTAGAGATGATTCTAAGAATACCCTGTATCTGCAGATGAACTCTCTGAGAGCTGAGGATACCGCTGTGTATTACTGTGCTAGACATGACAATTTTGGCAACTCTTATGTGTCTTGGTTTGCTTATTGGGGACAGGGAACACTGGTGACAGTGAGCTCTGGTGGAGGCGGTTCAGGCGGCGGAGGCAGCGGAGGTGGCGGGAGTGGAGGGGGTGGCTCTCAGACCGTGGTGACACAGGAGCCCAGCCTGACCGTGAGCCCCGGCGGCACCGTGACCCTGACCTGCGGCTCCTCCACAGGCGCCGTGACCACCTCCAACTACCCCAACTGGGTGCAGCAGAAGCCCGGCCAGGCCCCAAGGGGCCTGATCGGCGGCACCAATAAGAGGGCCCCCGGCGTGCCCGCTAGATTCTCTGGCTCTCTTCTGGGAGGAAAGGCTGCTCTGACACTGTCTGGAGCTCAGCCCGAGGATGAGGCTGAATACTATTGTGCTCTGTGGTATTCTGATCTGTGGGTGTTTGGCGGTGGAACTAAACTTACAGTTCTGGGCGGGGGCGGTAGCCAGGTGCAGCTGGTCCAGAGCGGAGCCGAGGTGAAGAAGCCCGGCGCCAGCGTGAAGGTGAGCTGCAAGGCCAGCGGCTACACTTTTACCTCTTACTACATTCACTGGGTGAGACAGGCTCCCGGCCAGTGCCTGGAGTGGATGGGATCCATCTATCCTGGAAATGTGAACACCAACTATAATGAGAAGTTTAAAGATAGAGTGACCCTGACCGTGGATACATCTATCTCTACCGCTTATATGGAGCTGTCTAGACTGAGATCCGATGACACAGCTGTGTATTATTGTACCAGATCTCATTACGGACTGGATTGGAATTTTGATGTGTGGGGCCAGGGCACCACAGTGACCGTGTCTTCTGGTGGGGGTGGTTCAGGGGGTGGTGGAAGTGGCGGTGGAGGGAGTGACAAGACCCACACATGTCCCCCCTGTCCCGCTCCTGAAGCTGCAGGAGCCCCTTCCGTGTTCCTGTTCCCCCCTAAGCCCAAGGACACCCTGATGATTTCCAGGACACCCGAGGTGACCTGTGTGGTGGTGGACGTCAGCCACGAGGACCCCGAGGTGAAATTCAACTGGTACGTCGATGGCGTGGAGGTGCACAACGCTAAGACCAAGCCCAGGGAGGAGCAGTACAATTCCACCTACAGGGTGGTGTCCGTGCTGACCGTCCTCCATCAGGACTGGCTGAACGGCAAAGAGTATAAGTGCAAGGTGAGCAACAAGGCCCTCCCTGCTCCCATCGAGAAGACCATCAGCAAAGCCAAGGGCCAGCCCAGGGAACCTCAAGTCTATACCCTGCCTCCCTGCAGGGATGAGCTGACCAAGAACCAAGTGAGCCTCTGGTGCCTCGTCAAGGGCTTCTATCCTTCCGATATTGCCGTCGAGTGGGAGTCCAACGGACAGCCCGAGAACAACTACAAGACAACACCCCCCGTGCTCGATTCCGATGGCAGCTTCTTCCTGTACTCCAAGCTGACCGTGGACAAGTCCAGATGGCAACAAGGCAACGTCTTCAGTTGCAGCGTCATGCATGAGGCCCTCCACAACCACTACACCCAGAAGAGCCTCTCCCTGAGCCCTGGAAAG

SEQ ID NO: 40 - protein, 451 aa, synthetic construct
  source 1..451: note = Amino acid sequence of 44H4-IgG1-Hole-HC
QVQLVQSGAEVKKPGASVKVSCKASGFNIKDTYIHWVRQAPGQGLEWMGRIDPANGYTKYGPRFQGRVTITADTSTSTVYMELSSLRSEDTAVYYCARNYGTSYPNAMDYWGQGTLVTVSSASTKGPSVFPLAPSSKSTSGGTAALGCLVKDYFPEPVTVSWNSGALTSGVHTFPAVLQSSGLYSLSSVVTVPSSSLGTQTYICNVNHKPSNTKVDKKVEPKSCDKTHTCPPCPAPEAAGAPSVFLFPPKPKDTLMISRTPEVTCVVVDVSHEDPEVKFNWYVDGVEVHNAKTKPREEQYNSTYRVVSVLTVLHQDWLNGKEYKCKVSNKALPAPIEKTISKAKGQPREPQVCTLPPSRDELTKNQVSLSCAVKGFYPSDIAVEWESNGQPENNYKTTPPVLDSDGSFFLVSKLTVDKSRWQQGNVFSCSVMHEALHNRFTQKSLSLSPGK

SEQ ID NO: 41 - protein, 1353 aa, synthetic construct
  source 1..1353: note = Nucleotide sequence of 44H4-IgG1-Hole-HC
CAGGTGCAGCTGGTGCAGTCTGGCGCTGAGGTGAAGAAGCCTGGCGCTTCTGTGAAGGTGTCTTGTAAGGCTTCTGGCTTTAATATCAAGGATACATATATCCATTGGGTGAGACAGGCCCCTGGCCAGGGCCTGGAGTGGATGGGCAGAATCGATCCAGCTAATGGCTACACCAAGTATGGCCCTAGATTTCAGGGAAGAGTGACCATCACAGCTGATACATCTACCTCCACCGTGTATATGGAGCTGTCCTCTCTGAGATCTGAGGATACAGCTGTGTATTATTGTGCTAGAAATTATGGCACATCTTACCCTAATGCTATGGATTACTGGGGACAGGGAACACTGGTGACAGTGAGCTCTGCTTCCACCAAAGGACCCAGCGTGTTTCCTCTGGCCCCTTCCAGCAAGAGCACCAGCGGAGGCACAGCTGCCCTGGGATGCCTGGTGAAGGACTATTTCCCTGAGCCCGTGACAGTCAGCTGGAACTCCGGCGCTCTGACCTCCGGCGTCCACACCTTTCCTGCCGTGCTGCAGAGCAGCGGCCTGTACAGCCTGTCCAGCGTGGTGACCGTGCCTAGCTCCAGCCTGGGCACCCAGACCTACATCTGCAACGTGAACCACAAGCCCTCCAACACCAAGGTGGACAAGAAGGTGGAGCCTAAGAGCTGTGACAAGACCCACACATGCCCTCCTTGTCCTGCTCCTGAAGCCGCCGGCGCACCTTCCGTGTTCCTGTTCCCCCCTAAGCCCAAGGATACCCTCATGATTTCCAGGACCCCCGAAGTGACCTGCGTGGTGGTCGATGTGAGCCACGAAGACCCTGAAGTGAAGTTCAACTGGTACGTGGACGGCGTCGAGGTCCACAACGCCAAAACCAAGCCCAGGGAGGAGCAGTACAATAGCACCTACCGGGTGGTGAGCGTGCTGACCGTGCTGCACCAGGACTGGCTGAACGGCAAGGAGTACAAGTGTAAGGTCAGCAACAAGGCCCTCCCTGCCCCCATCGAGAAGACCATTTCCAAGGCTAAGGGACAGCCTCGGGAACCCCAAGTGTGCACCCTGCCTCCTAGCAGGGATGAGCTGACCAAGAACCAGGTGAGCCTGAGCTGTGCTGTGAAGGGCTTCTACCCTTCCGACATCGCTGTCGAGTGGGAGAGCAACGGCCAGCCCGAGAATAACTACAAGACAACCCCCCCCGTGCTCGACAGCGATGGCAGCTTCTTTCTGGTGTCCAAGCTCACCGTGGACAAGTCCAGGTGGCAGCAGGGCAACGTCTTCTCCTGCTCCGTCATGCACGAGGCCCTGCACAACCGCTTCACACAGAAGTCCCTGTCCCTGTCCCCTGGAAAG

SEQ ID NO: 42 - protein, 744 aa, synthetic construct
  source 1..744: note = Amino acid sequence of CD28-44-SP34-2ScFv-IgG1-Knob-HC
DIQMTQSPSSLSASVGDRVTITCHASQNIYVWLNWYQQKPGKAPKLLIYKASNLHTGVPSRFSGSGSGTDFTLTISSLQPEDFATYYCQQGQTYPYTFGCGTKVEIKGGGGSGGGGSGGGGSGGGGSQVQLVQSGAEVKKPGASVKVSCKASGYTFTSYYIHWVRQAPGQCLEWMGSIYPGNVNTNYNEKFKDRVTLTVDTSISTAYMELSRLRSDDTAVYYCTRSHYGLDWNFDVWGQGTTVTVSSGGGSGGGSQTVVTQEPSLTVSPGGTVTLTCGSSTGAVTTSNYPNWVQQKPGQAPRGLIGGTNKRAPGVPARFSGSLLGGKAALTLSGAQPEDEAEYYCALWYSDLWVFGGGTKLTVLGGGGSGGGGSGGGGSGGGGSEVQLVESGGGLVQPGGSLRLSCAASGFTFSTYAMNWVRQAPGKGLEWVSRIRSKYNNYATYYADSVKDRFTISRDDSKNTLYLQMNSLRAEDTAVYYCARHDNFGNSYVSWFAYWGQGTLVTVSSGGGSGGGSDKTHTCPPCPAPEAAGAPSVFLFPPKPKDTLMISRTPEVTCVVVDVSHEDPEVKFNWYVDGVEVHNAKTKPREEQYNSTYRVVSVLTVLHQDWLNGKEYKCKVSNKALPAPIEKTISKAKGQPREPQVYTLPPCRDELTKNQVSLWCLVKGFYPSDIAVEWESNGQPENNYKTTPPVLDSDGSFFLYSKLTVDKSRWQQGNVFSCSVMHEALHNHYTQKSLSLSPGK

SEQ ID NO: 43 - protein, 2232 aa, synthetic construct
  source 1..2232: note = Nucleotide sequence of CD28-44-SP34-2ScFv-IgG1-Knob-HC
GACATCCAGATGACCCAGAGTCCCAGCAGCCTGTCTGCTTCTGTGGGAGATAGAGTGACAATTACATGTCATGCTTCTCAGAATATCTACGTGTGGCTGAACTGGTACCAGCAGAAACCTGGAAAGGCTCCTAAGCTGCTGATCTACAAGGCTTCTAACCTGCACACAGGCGTGCCTTCTAGATTTTCTGGATCTGGCTCCGGAACAGATTTTACTCTGACCATCTCTAGCCTGCAGCCAGAAGATTTTGCCACCTATTATTGTCAGCAGGGACAGACCTACCCTTACACATTTGGCTGCGGCACAAAGGTGGAGATCAAGGGTGGAGGCGGTTCAGGCGGCGGAGGCAGCGGAGGTGGCGGGAGTGGAGGGGGTGGCTCTCAGGTGCAGCTGGTCCAGAGCGGAGCCGAGGTGAAGAAGCCCGGCGCCAGCGTGAAGGTGAGCTGCAAGGCCAGCGGCTACACTTTTACCTCTTACTACATTCACTGGGTGAGACAGGCTCCCGGCCAGTGCCTGGAGTGGATGGGATCTATCTATCCTGGAAATGTGAACACCAACTATAATGAGAAGTTTAAAGATAGAGTGACCCTGACCGTGGATACATCTATCTCTACCGCTTATATGGAGCTGTCTAGACTGAGATCCGATGACACAGCTGTGTATTATTGTACCAGATCTCATTACGGACTGGATTGGAATTTTGATGTGTGGGGCCAGGGCACCACAGTGACCGTGTCTTCTGGGGGCGGTAGCGGGGGCGGGTCTCAGACCGTGGTGACACAGGAGCCCAGCCTGACCGTGAGCCCCGGCGGCACCGTGACCCTGACCTGCGGCTCCTCCACCGGCGCCGTGACCACCTCCAACTACCCCAACTGGGTGCAGCAGAAGCCCGGCCAGGCCCCAAGGGGCCTGATCGGCGGCACCAATAAGAGGGCCCCCGGCGTGCCCGCTAGATTCTCTGGCTCTCTTCTGGGAGGAAAGGCTGCTCTGACACTGTCTGGAGCTCAGCCCGAGGATGAGGCTGAATACTATTGTGCTCTGTGGTATTCTGATCTGTGGGTGTTTGGCGGTGGAACTAAACTTACAGTTCTGGGTGGGGGTGGTTCAGGGGGTGGTGGAAGTGGCGGTGGAGGGAGTGGTGGAGGCGGTAGCGAGGTGCAGCTGGTGGAGTCTGGCGGCGGCCTGGTGCAGCCTGGCGGCTCTCTGAGACTGTCTTGTGCTGCTTCTGGCTTTACCTTTTCTACCTATGCTATGAATTGGGTGAGACAGGCTCCTGGCAAGGGCCTGGAGTGGGTGTCTAGAATCAGATCTAAGTATAATAATTACGCTACCTATTATGCTGATTCTGTGAAGGACAGATTCACAATCTCTAGAGATGATTCTAAGAATACCCTGTATCTGCAGATGAACTCTCTGAGAGCTGAGGATACCGCTGTGTATTACTGTGCTAGACATGACAATTTTGGCAACTCTTATGTGTCTTGGTTTGCTTATTGGGGACAGGGAACACTGGTGACAGTGAGCTCTGGCGGGGGATCAGGAGGTGGCAGTGACAAGACCCACACATGTCCCCCCTGTCCCGCTCCTGAAGCTGCAGGAGCCCCTTCCGTGTTCCTGTTCCCCCCTAAGCCCAAGGACACCCTGATGATTTCCAGGACACCCGAGGTGACCTGTGTGGTGGTGGACGTCAGCCACGAGGACCCCGAGGTGAAATTCAACTGGTACGTCGATGGCGTGGAGGTGCACAACGCTAAGACCAAGCCCAGGGAGGAGCAGTACAATTCCACCTACAGGGTGGTGTCCGTGCTGACCGTCCTCCATCAGGACTGGCTGAACGGCAAAGAGTATAAGTGCAAGGTGAGCAACAAGGCCCTCCCTGCTCCCATCGAGAAGACCATCAGCAAAGCCAAGGGCCAGCCCAGGGAACCTCAAGTCTATACCCTGCCTCCCTGCAGGGATGAGCTGACCAAGAACCAAGTGAGCCTCTGGTGCCTCGTCAAGGGCTTCTATCCTTCCGATATTGCCGTCGAGTGGGAGTCCAACGGACAGCCCGAGAACAACTACAAGACAACACCCCCCGTGCTCGATTCCGATGGCAGCTTCTTCCTGTACTCCAAGCTGACCGTGGACAAGTCCAGATGGCAACAAGGCAACGTCTTCAGTTGCAGCGTCATGCATGAGGCCCTCCACAACCACTACACCCAGAAGAGCCTCTCCCTGAGCCCTGGAAAG

SEQ ID NO: 44 - protein, 227 aa, synthetic construct
  source 1..227: note = Amino acid sequence of IgG1-Knob-HC
DKTHTCPPCPAPEAAGAPSVFLFPPKPKDTLMISRTPEVTCVVVDVSHEDPEVKFNWYVDGVEVHNAKTKPREEQYNSTYRVVSVLTVLHQDWLNGKEYKCKVSNKALPAPIEKTISKAKGQPREPQVYTLPPCRDELTKNQVSLWCLVKGFYPSDIAVEWESNGQPENNYKTTPPVLDSDGSFFLYSKLTVDKSRWQQGNVFSCSVMHEALHNHYTQKSLSLSPGK

SEQ ID NO: 45 - protein, 227 aa, synthetic construct
  source 1..227: note = Amino acid sequence of IgG1-Hole-HC
DKTHTCPPCPAPEAAGAPSVFLFPPKPKDTLMISRTPEVTCVVVDVSHEDPEVKFNWYVDGVEVHNAKTKPREEQYNSTYRVVSVLTVLHQDWLNGKEYKCKVSNKALPAPIEKTISKAKGQPREPQVCTLPPSRDELTKNQVSLSCAVKGFYPSDIAVEWESNGQPENNYKTTPPVLDSDGSFFLVSKLTVDKSRWQQGNVFSCSVMHEALHNRFTQKSLSLSPGK

SEQ ID NO: 46 - protein, 271 aa, synthetic construct
  source 1..271: note = Amino acid sequence of MUC17-His
RTTTCFGDGCQNTASRCKNGGTWDGLKCQCPNLYYGELCEEVVSSIDIGPPETISAQMELTVTVTSVKFTEELKNHSSQEFQEFKQTFTEQMNIVYSGIPEYVGVNITKLRLGSVVVEHDVLLRTKYTPEYKTVLDNATEVVKEKITKVTTQQIMINDICSDMMCFNTTGTQVQNITVTQYDPEEDCRKMAKEYGDYFVVEYRDQKPYCISPCEPGFSVSKNCNLGKCQMSLSGPQCLCVTTETHWYSGETCNQGTQKSLGGGGSHHHHHH

SEQ ID NO: 47 - protein, 145 aa, synthetic construct
  source 1..145: note = Amino acid sequence of CD28-His
NKILVKQSPMLVAYDNAVNLSCKYSYNLFSREFRASLHKGLDSAVEVCVVYGNYSQQLQVYSKTGFNCDGKLGNESVTFYLQNLYVNQTDIYFCKIEVMYPPPYLDNEKSNGTIIHVKGKHLCPSPLFPGPSKPGGGGSHHHHHH

SEQ ID NO: 48 - protein, 574 aa, synthetic construct
  source 1..574: note = Amino acid sequence of CD28-CD3-CODV-IgG1-Knob-HC
QVQLVQSGAEVVKPGASVKVSCKASGYTFTSYYIHWVRQAPGQGLEWIGSIYPGNVNTNYAQKFQGRATLTVDTSISTAYMELSRLRSDDTAVYYCTRSHYGLDWNFDVWGKGTTVTVSSSQVQLVESGGGVVQPGRSLRLSCAASGFTFTKAWMHWVRQAPGKQLEWVAQIKDKSNSYATYYADSVKGRFTISRDDSKNTLYLQMNSLRAEDTAVYYCRGVYYALSPFDYWGQGTLVTVSSRTASTKGPSVFPLAPSSKSTSGGTAALGCLVKDYFPEPVTVSWNSGALTSGVHTFPAVLQSSGLYSLSSVVTVPSSSLGTQTYICNVNHKPSNTKVDKKVEPKSCDKTHTCPPCPAPEAAGAPSVFLFPPKPKDTLMISRTPEVTCVVVDVSHEDPEVKFNWYVDGVEVHNAKTKPREEQYNSTYRVVSVLTVLHQDWLNGKEYKCKVSNKALPAPIEKTISKAKGQPREPQVYTLPPCRDELTKNQVSLWCLVKGFYPSDIAVEWESNGQPENNYKTTPPVLDSDGSFFLYSKLTVDKSRWQQGNVFSCSVMHEALHNHYTQKSLSLSPGK

SEQ ID NO: 49 - protein, 338 aa, synthetic construct
  source 1..338: note = Amino acid sequence of CD3-CD28-CODV-LC
DIVMTQTPLSLSVTPGQPASISCKSSQSLVHNNANTYLSWYLQKPGQSPQSLIYKVSNRFSGVPDRFSGSGSGTDFTLKISRVEAEDVGVYYCGQGTQYPFTFGSGTKVEIKGQPKAAPDIQMTQSPSSLSASVGDRVTITCQASQNIYVWLNWYQQKPGKAPKLLIYKASNLHTGVPSRFSGSGSGTDFTLTISSLQPEDIATYYCQQGQTYPYTFGQGTKLEIKTKGPSRTVAAPSVFIFPPSDEQLKSGTASVVCLLNNFYPREAKVQWKVDNALQSGNSQESVTEQDSKDSTYSLSSTLTLSKADYEKHKVYACEVTHQGLSSPVTKSFNRGEC

SEQ ID NO: 50 - protein, 120 aa, synthetic construct
  source 1..120: note = Amino acid sequence of VH of modified Anti-CD28
QVQLVQSGAEVKKPGASVKVSCKASGYTFTSYYIHWVRQAPGQGLEWMGSIYPGNVNTNYNEKFKDRVTLTVDTSISTAYMELSRLRSDDTAVYYCTRSHYGLDWNFDVWGQGTTVTVSS

SEQ ID NO: 51 - protein, 14 aa, synthetic construct
  source 1..14: note = H-CDR3 of the SP34 humanized antibody
HDNFGNSYVSWFAY

SEQ ID NO: 52 - protein, 9 aa, synthetic construct
  source 1..9: note = L-CDR3 of the SP34 humanized antibody
ALWYSDLWV

SEQ ID NO: 53 - protein, 17 aa, synthetic construct
  source 1..17: note = H-CDR2 of Anti-CD28 humanized antibody
SIYPGNVNTNYNEKFKD